European Patent Specification EP 4 047 017 B1, published March 4, 2026. Title: MONOCLONAL ANTIBODY, MEASUREMENT REAGENT FOR CYTOKERATIN 18 FRAGMENT, REAGENT KIT, AND MEASUREMENT METHOD. Applicant: Sysmex Corporation. The sequence listing filed with the application follows.

SEQUENCE LISTING (48 sequences)

SEQ ID NO: 1 - protein, 5 aa, Mus musculus
SFGMH

SEQ ID NO: 2 - protein, 17 aa, Mus musculus
YISSGSTTIYYADTVKG

SEQ ID NO: 3 - protein, 12 aa, Mus musculus
RGMITTGAWFAY

SEQ ID NO: 4 - protein, 11 aa, Mus musculus
RASQRIGTSIH

SEQ ID NO: 5 - protein, 7 aa, Mus musculus
YASESIS

SEQ ID NO: 6 - protein, 9 aa, Mus musculus
QQSYIWPFT

SEQ ID NO: 7 - protein, 121 aa, Mus musculus
DVQLVESGGGLVQPGGSRKLSCAASGFTFSSFGMHWVRQAPEKGLEWVAYISSGSTTIYYADTVKGRFTISRDNPKNTLFLQMTSLRSEDTAMYYCARRGMITTGAWFAYWGQGTLVTVSA

SEQ ID NO: 8 - protein, 107 aa, Mus musculus
DILLTQSPAILSVSPGERVSFSCRASQRIGTSIHWYQQRTNGSPRLLIKYASESISGIPSRFSGSGSGTDFTLSINSVESEDIADYYCQQSYIWPFTFGSGTKLEIK

SEQ ID NO: 9 - protein, 430 aa, Homo sapiens
MSFTTRSTFSTNYRSLGSVQAPSYGARPVSSAASVYAGAGGSGSRISVSRSTSFRGGMGSGGLATGIAGGLAGMGGIQNEKETMQSLNDRLASYLDRVRSLETENRRLESKIREHLEKKGPQVRDWSHYFKIIEDLRAQIFANTVDNARIVLQIDNARLAADDFRVKYETELAMRQSVENDIHGLRKVIDDTNITRLQLETEIEALKEELLFMKKNHEEEVKGLQAQIASSGLTVEVDAPKSQDLAKIMADIRAQYDELARKNREELDKYWSQQIEESTTVVTTQSAEVGAAETTLTELRRTVQSLEIDLDSMRNLKASLENSLREVEARYALQMEQLNGILLHLESELAQTRAEGQRQAQEYEALLNIKVKLEAEIATYRRLLEDGEDFNLGDALDSSNSMQTIQKTTTRRIVDGKVVSETNDTKVLRH

SEQ ID NO: 10 - protein, 17 aa, Artificial Sequence
  synthetic
RRLLEDGEDFNLGDALD

SEQ ID NO: 11 - protein, 16 aa, Artificial Sequence
  synthetic
RRLLEDGEDFNLGDAL

SEQ ID NO: 12 - protein, 18 aa, Artificial Sequence
  synthetic
APKSQDLAKIMADIRAQY

SEQ ID NO: 13 - protein, 18 aa, Artificial Sequence
  synthetic
LAKIMADIRAQYDELARK

SEQ ID NO: 14 - protein, 18 aa, Artificial Sequence
  synthetic
DIRAQYDELARKNREELD

SEQ ID NO: 15 - protein, 18 aa, Artificial Sequence
  synthetic
DELARKNREELDKYWSQQ

SEQ ID NO: 16 - protein, 18 aa, Artificial Sequence
  synthetic
NREELDKYWSQQIEESTT

SEQ ID NO: 17 - protein, 18 aa, Artificial Sequence
  synthetic
KYWSQQIEESTTVVTTQS

SEQ ID NO: 18 - protein, 18 aa, Artificial Sequence
  synthetic
IEESTTVVTTQSAEVGAA

SEQ ID NO: 19 - protein, 18 aa, Artificial Sequence
  synthetic
VVTTQSAEVGAAETTLTE

SEQ ID NO: 20 - protein, 18 aa, Artificial Sequence
  synthetic
AEVGAAETTLTELRRTVQ

SEQ ID NO: 21 - protein, 18 aa, Artificial Sequence
  synthetic
ETTLTELRRTVQSLEIDL

SEQ ID NO: 22 - protein, 18 aa, Artificial Sequence
  synthetic
LRRTVQSLEIDLDSMRNL

SEQ ID NO: 23 - protein, 18 aa, Artificial Sequence
  synthetic
SLEIDLDSMRNLKASLEN

SEQ ID NO: 24 - protein, 18 aa, Artificial Sequence
  synthetic
DSMRNLKASLENSLREVE

SEQ ID NO: 25 - protein, 18 aa, Artificial Sequence
  synthetic
KASLENSLREVEARYALQ

SEQ ID NO: 26 - protein, 18 aa, Artificial Sequence
  synthetic
SLREVEARYALQMEQLNG

SEQ ID NO: 27 - protein, 18 aa, Artificial Sequence
  synthetic
ARYALQMEQLNGILLHLE

SEQ ID NO: 28 - protein, 18 aa, Artificial Sequence
  synthetic
MEQLNGILLHLESELAQT

SEQ ID NO: 29 - protein, 18 aa, Artificial Sequence
  synthetic
ILLHLESELAQTRAEGQR

SEQ ID NO: 30 - protein, 18 aa, Artificial Sequence
  synthetic
SELAQTRAEGQRQAQEYE

SEQ ID NO: 31 - protein, 18 aa, Artificial Sequence
  synthetic
RAEGQRQAQEYEALLNIK

SEQ ID NO: 32 - protein, 18 aa, Artificial Sequence
  synthetic
QAQEYEALLNIKVKLEAE

SEQ ID NO: 33 - protein, 18 aa, Artificial Sequence
  synthetic
ALLNIKVKLEAEIATYRR

SEQ ID NO: 34 - protein, 18 aa, Artificial Sequence
  synthetic
VKLEAEIATYRRLLEDGE

SEQ ID NO: 35 - protein, 18 aa, Artificial Sequence
  synthetic
IATYRRLLEDGEDFNLGD

SEQ ID NO: 36 - protein, 15 aa, Artificial Sequence
  synthetic
LLEDGEDFNLGDALD

SEQ ID NO: 37 - protein, 304 aa, Artificial Sequence
  synthetic
SHYFKIIEDLRAQIFANTVDNARIVLQIDNARLAADDFRVKYETELAMRQSVENDIHGLRKVIDDTNITRLQLETEIEALKEELLFMKKNHEEEVKGLQAQIASSGLTVEVDAPKSQDLAKIMADIRAQYDELARKNREELDKYWSQQIEESTTVVTTQSAEVGAAETTLTELRRTVQSLEIDLDSMRNLKASLENSLREVEARYALQMEQLNGILLHLESELAQTRAEGQRQAQEYEALLNIKVKLEAEIATYRRLLEDGEDFNLGDALDSSNSMQTIQKTTTRRIVDGKVVSETNDTKVLRH

SEQ ID NO: 38 - protein, 158 aa, Artificial Sequence
  synthetic
APKSQDLAKIMADIRAQYDELARKNREELDKYWSQQIEESTTVVTTQSAEVGAAETTLTELRRTVQSLEIDLDSMRNLKASLENSLREVEARYALQMEQLNGILLHLESELAQTRAEGQRQAQEYEALLNIKVKLEAEIATYRRLLEDGEDFNLGDAL

SEQ ID NO: 39 - protein, 159 aa, Artificial Sequence
  synthetic
APKSQDLAKIMADIRAQYDELARKNREELDKYWSQQIEESTTVVTTQSAEVGAAETTLTELRRTVQSLEIDLDSMRNLKASLENSLREVEARYALQMEQLNGILLHLESELAQTRAEGQRQAQEYEALLNIKVKLEAEIATYRRLLEDGEDFNLGDALD

SEQ ID NO: 40 - protein, 8 aa, Mus musculus
GYTFTNYT

SEQ ID NO: 41 - protein, 8 aa, Mus musculus
INPSSGYT

SEQ ID NO: 42 - protein, 8 aa, Mus musculus
ARQIPFAY

SEQ ID NO: 43 - protein, 10 aa, Mus musculus
ESVDSYGISF

SEQ ID NO: 44 - protein, 9 aa, Mus musculus
QQSKEVPWT

SEQ ID NO: 45 - protein, 115 aa, Mus musculus
QVHLQQSAAELARPGASVKMSCKASGYTFTNYTIHWIKQRPGQGLEWIGYINPSSGYTDYNQNFKDKTTLTADKSSTTVYMQLSSLTSEDSAVYYCARQIPFAYWGQGTLVTVSA

SEQ ID NO: 46 - protein, 111 aa, Mus musculus
DIVLTQSPASLAVSLGQRATISCRASESVDSYGISFMNWFQQKPGQPPKLLIYAASNQGSGVPARFSGSGSGTDFSLNIHPMEVDDTAMYFCQQSKEVPWTFGGGTKLEIK

SEQ ID NO: 47 - protein, 137 aa, Artificial Sequence
  synthetic
RKNREELDKYWSQQIEESTTVVTTQSAEVGAAETTLTELRRTVQSLEIDLDSMRNLKASLENSLREVEARYALQMEQLNGILLHLESELAQTRAEGQRQAQEYEALLNIKVKLEAEIATYRRLLEDGEDFNLGDALD

SEQ ID NO: 48 - protein, 157 aa, Artificial Sequence
  synthetic
KSQDLAKIMADIRAQYDELARKNREELDKYWSQQIEESTTVVTTQSAEVGAAETTLTELRRTVQSLEIDLDSMRNLKASLENSLREVEARYALQMEQLNGILLHLESELAQTRAEGQRQAQEYEALLNIKVKLEAEIATYRRLLEDGEDFNLGDALD